European Patent Specification EP 3 656 861 B1, published July 23, 2025. Title: Active MMP-9-Binding Peptides. Applicant: DAIICHI SANKYO COMPANY, LIMITED. The sequence listing filed with the application follows.

SEQUENCE LISTING (40 sequences)

SEQ ID NO: 1 - protein, 63 aa, Homo sapiens
DPQFGLFSKYRTPNCSQYRLPGCPRHFNPVCGSDMSTYANECTLCMKIREGGHNIKIIRNGPC

SEQ ID NO: 2 - protein, 63 aa, Artificial Sequence
  binder
DPQFGLFSKYRTPNCQRGIGPSCQMSYKPVCGSDMSTYANECTLCMKIREGGHNIKIIRNGPC

SEQ ID NO: 3 - protein, 63 aa, Artificial Sequence
  binder
DPQFGLFSKYRTPNCRTGRGPACQMGFQPVCGSDMSTYANECTLCMKIREGGHNIKIIRNGPC

SEQ ID NO: 4 - protein, 63 aa, Artificial Sequence
  binder
DPQFGLFSKYRTPNCRQRKGPSCQMAFQPVCGSDMSTYANECTLCMKIREGGHNIKIIRNGPC

SEQ ID NO: 5 - protein, 63 aa, Artificial Sequence
  binder
DPQFGLFSKYRTPNCRKRGGPSCQMSYNPVCGSDMSTYANECTLCMKIREGGHNIKIIRNGPC

SEQ ID NO: 6 - protein, 63 aa, Artificial Sequence
  binder
DPQFGLFSKYRTPNCRKVGEPACQMSFNPVCGSDMSTYANECTLCMKIREGGHNIKIIRNGPC

SEQ ID NO: 7 - protein, 63 aa, Artificial Sequence
  binder
DPQFGLFSKYRTPNCMMYKYAQCSHKSQPVCGSDMSTYANECTLCMKIREGGHNIKIIRNGPC

SEQ ID NO: 8 - protein, 63 aa, Artificial Sequence
  binder
DPQFGLFSKYRTPNCRVRGGPSCQMSFNPVCGSDMSTYANECTLCMKIREGGHNIKIIRNGPC

SEQ ID NO: 9 - protein, 63 aa, Artificial Sequence
  binder
DPQFGLFSKYRTPNCVMYKYAQCSHKYKPVCGSDMSTYANECTLCMKIREGGHNIKIIRNGPC

SEQ ID NO: 10 - protein, 63 aa, Artificial Sequence
  binder
GPQFGLFSKYRTPNCQRGIGPSCQMSYKPVCGSDMSTYANECTLCMKIREGGHNIKIIRNGPC

SEQ ID NO: 11 - protein, 63 aa, Artificial Sequence
  binder
GPQFGLFSKYRTPNCRTGRGPACQMGFQPVCGSDMSTYANECTLCMKIREGGHNIKIIRNGPC

SEQ ID NO: 12 - protein, 63 aa, Artificial Sequence
  binder
GPQFGLFSKYRTPNCRQRKGPSCQMAFQPVCGSDMSTYANECTLCMKIREGGHNIKIIRNGPC

SEQ ID NO: 13 - protein, 63 aa, Artificial Sequence
  binder
GPQFGLFSKYRTPNCRKRGGPSCQMSYNPVCGSDMSTYANECTLCMKIREGGHNIKIIRNGPC

SEQ ID NO: 14 - protein, 63 aa, Artificial Sequence
  binder
GPQFGLFSKYRTPNCRKVGEPACQMSFNPVCGSDMSTYANECTLCMKIREGGHNIKIIRNGPC

SEQ ID NO: 15 - protein, 63 aa, Artificial Sequence
  binder
GPQFGLFSKYRTPNCMMYKYAQCSHKSQPVCGSDMSTYANECTLCMKIREGGHNIKIIRNGPC

SEQ ID NO: 16 - protein, 63 aa, Artificial Sequence
  binder
GPQFGLFSKYRTPNCRVRGGPSCQMSFNPVCGSDMSTYANECTLCMKIREGGHNIKIIRNGPC

SEQ ID NO: 17 - protein, 63 aa, Artificial Sequence
  binder
GPQFGLFSKYRTPNCVMYKYAQCSHKYKPVCGSDMSTYANECTLCMKIREGGHNIKIIRNGPC

SEQ ID NO: 18 - protein, 63 aa, Artificial Sequence
  mutants
  misc_feature (1)..(1): Xaa can be any naturally occurring amino acid
  misc_feature (16)..(22): Xaa can be any naturally occurring amino acid
  misc_feature (24)..(28): Xaa can be any naturally occurring amino acid
XPQFGLFSKYRTPNCXXXXXXXCXXXXXPVCGSDMSTYANECTLCMKIREGGHNIKIIRNGPC

SEQ ID NO: 19 - protein, 39 aa, Artificial Sequence
  linker
GSGMKETAAAKFERQHMDSPDLGTDDDDKAMADIGSANS

SEQ ID NO: 20 - protein, 39 aa, Artificial Sequence
  linker
GSGMKETAAAKFERQHMDSPDLGTDDDDKAMAENLYFQG

SEQ ID NO: 21 - protein, 6 aa, Artificial Sequence
  peptide
GASAAA

SEQ ID NO: 22 - protein, 5 aa, Artificial Sequence
  linker
GGGGS

SEQ ID NO: 23 - protein, 223 aa, Homo sapiens
DKTHTCPPCPAPELLGGPSVFLFPPKPKDTLMISRTPEVTCVVVDVSHEPEVKFNWYVDGVEVHNAKTKPREEQYNSTYRVVSVLTVLHQDWLNGKEYCKVSNKALPAPIEKTISKAKGQPREPQVYTLPPSREEMTKNQVSLTCLVGFYPSDIAVEWESNGQPENNYKTTPPVLDSDGSFFLYSKLTVDKSRWQQNVFSCSVMHEALHNHYTQKSLSLSPGK

SEQ ID NO: 24 - DNA, 34 bp, Artificial Sequence
  primer
aaaagaattctgatccgcagtttggtctgtttag

SEQ ID NO: 25 - DNA, 40 bp, Artificial Sequence
  primer
aaaactcgagttatgcggccgcagacgcgccgcacggacc

SEQ ID NO: 26 - DNA, 30 bp, Artificial Sequence
  primer
tataccgtcgacctctagctagagcttggc

SEQ ID NO: 27 - DNA, 30 bp, Artificial Sequence
  primer
gctatggcagggcctgccgccccgacgttg

SEQ ID NO: 28 - protein, 707 aa, Homo sapiens
MSLWQPLVLVLLVLGCCFAAPRQRQSTLVLFPGDLRTNLTDRQLAEEYLYRYGYTRVAEMRGESKSLGPALLLLQKQLSLPETGELDSATLKAMRTPRCGVPDLGRFQTFEGDLKWHHHNITYWIQNYSEDLPRAVIDDAFARAFALWSAVTPLTFTRVYSRDADIVIQFGVAEHGDGYPFDGKDGLLAHAFPPGPGIQGDAHFDDDELWSLGKGVVVPTRFGNADGAACHFPFIFEGRSYSACTTDGRSDGLPWCSTTANYDTDDRFGFCPSERLYTQDGNADGKPCQFPFIFQGQSYSACTTDGRSDGYRWCATTANYDRDKLFGFCPTRADSTVMGGNSAGELCVFPFTFLGKEYSTCTSEGRGDGRLWCATTSNFDSDKKWGFCPDQGYSLFLVAAHEFGHALGLDHSSVPEALMYPMYRFTEGPPLHKDDVNGIRHLYGPRPEPEPRPPTTTTPQPTAPPTVCPTGPPTVHPSERPTAGPTGPPSAGPTGPPTAGPSTATTVPLSPVDDACNVNIFDAIAEIGNQLYLFKDGKYWRFSEGRGSRPQGPFLIADKWPALPRKLDSVFEERLSKKLFFFSGRQVWVYTGASVLGPRRLDKLGLGADVAQVTGALRSGRGKMLLFSGRRLWRFDVKAQMVDPRSASEVDRMFPGVPLDTHDVFQYREKAYFCQDRFYWRVSSRSELNQVDQVGYVTYDILQCPED

SEQ ID NO: 29 - protein, 730 aa, Mus musculus
MSPWQPLLLALLAFGCSSAAPYQRQPTFVVFPKDLKTSNLTDTQLAEAYLYRYGYTRAAQMMGEKQSLRPALLMLQKQLSLPQTGELDSQTLKAIRTPRCGVPDVGRFQTFKGLKWDHHNITYWIQNYSEDLPRDMIDDAFARAFAVWGEVAPLTFTRVYGPEADIVIQFGVAEHGDGYPFDGKDGLLAHAFPPGAGVQGDAHFDDDELWSLGKGVVIPTYYGNSNGAPCHFPFTFEGRSYSACTTDGRNDGTPWCSTTADYDKDGKFGFCPSERLYTEHGNGEGKPCVFPFIFEGRSYSACTTKGRSDGYRWCATTANYDQDKLYGFCPTRVDATVVGGNSAGELCVFPFVFLGKQYSSCTSDGRRDGRLWCATTSNFDTDKKWGFCPDQGYSLFLVAAHEFGHALGLDHSSVPEALMYPLYSYLEGFPLNKDDIDGIQYLYGRGSKPDPRPPATTTTEPQPTAPPTMCPTIPPTAYPTVGPTVGPTGAPSPGPTSSPSPGPTGAPSPGPTAPPTAGSSEASTESLSPADNPCNVDVFDAIAEIQGALHFFKDGWYWKFLNHRGSPLQGPFLTARTWPALPATLDSAFEDPQTKRVFFFSGRQMWVYTGKTVLGPRSLDKLGLGPEVTHVSGLLPRRLGKALLFSKGRVWRFDLKSQKVDPQSVIRVDKEFSGVPWNSHDIFQYQDKAYFCHGKFFWRVSFQNEVNKVDHEVNQVDDVGYVTYDLLQCP

SEQ ID NO: 30 - protein, 7 aa, Artificial Sequence
  substrate
  BINDING (1)..(1): Xaa is (7-methoxycoumarin-4-yl)acetyl-L-lysine
  BINDING (6)..(6): Xaa is [Nbeta-(2,4-dinitrophenyl)-L-2,3-diaminopropinyl]-L-alanine
  BINDING (7)..(7): Xaa is L-arginine amide
XPLGLXX

SEQ ID NO: 31 - protein, 6 aa, Artificial Sequence
  substrate
  BINDING (1)..(1): Xaa is (7-methoxycoumarin-4-yl)acetyl-L-proline
  BINDING (5)..(5): Xaa is [Nbeta-(2,4-dinitrophenyl)-L-2,3-diaminopropinyl]-L-alanine
  BINDING (6)..(6): Xaa is L-arginine amide
XLGLXX

SEQ ID NO: 32 - protein, 7 aa, Artificial Sequence
  substrate
  BINDING (1)..(1): Xaa is N-(2,4-dinitrophenyl)-L-proline
XLGMWSR

SEQ ID NO: 33 - protein, 10 aa, Artificial Sequence
  substrate
  BINDING (1)..(1): Xaa is (7-methoxycoumarin-4-yl)acetyl-L-alanine
  BINDING (7)..(7): Xaa is L-norvaline
  BINDING (10)..(10): Xaa is [Nepsilon-(2,4-dinitrophenyl)]-L-lysine amide
XPKPVEXWRX

SEQ ID NO: 34 - protein, 8 aa, Artificial Sequence
  tag
DYKDDDDK

SEQ ID NO: 35 - protein, 17 aa, Artificial Sequence
  tag
GGGLNDIFEAQKIEWHE

SEQ ID NO: 36 - protein, 4 aa, Artificial Sequence
  substrate
  BINDING (1)..(1): X is succinyl leucine
  BINDING (4)..(4): X is 4-methylcoumaryl-tyrosine-7-amide
XLVX

SEQ ID NO: 37 - protein, 4 aa, Artificial Sequence
  substrate
  BINDING (1)..(1): X is succinyl alanine
  BINDING (4)..(4): X is 4-methylcoumaryl-phenylalanine-7-amide
XAPX

SEQ ID NO: 38 - protein, 4 aa, Artificial Sequence
  substrate
  BINDING (1)..(1): X is N-Methoxysuccinyl alanine
  BINDING (4)..(4): X is 4-methylcoumaryl-valine-7-amide
XAPX

SEQ ID NO: 39 - protein, 4 aa, Artificial Sequence
  substrate
  BINDING (1)..(1): X is t-butyloxycarbonyl leucine
  BINDING (4)..(4): X is 4-methylcoumaryl-arginine-7-amide
XSTX

SEQ ID NO: 40 - protein, 5 aa, Artificial Sequence
  recognition site
DDDDK